European Patent Specification EP 3 521 419 B1, published March 18, 2026. Title: A method for producing a somatic cell, and a somatic cell and a composition. Applicant: Kyoto Prefectural Public University Corporation. The sequence listing filed with the application follows.

SEQUENCE LISTING (14 sequences)

SEQ ID NO: 1 - DNA, 23 bp, Artificial Sequence
  Description of Artificial Sequence: Synthetic DNA
actacggggttatcacctgtgag

SEQ ID NO: 2 - DNA, 22 bp, Artificial Sequence
  Description of Artificial Sequence: Synthetic DNA
gtgcaggagtaggccacattac

SEQ ID NO: 3 - DNA, 20 bp, Artificial Sequence
  Description of Artificial Sequence: Synthetic DNA
tctacgacacggtccaggag

SEQ ID NO: 4 - DNA, 22 bp, Artificial Sequence
  Description of Artificial Sequence: Synthetic DNA
gaatactgccactcctccagtc

SEQ ID NO: 5 - DNA, 19 bp, Artificial Sequence
  Description of Artificial Sequence: Synthetic DNA
agcaggaatggctcgagac

SEQ ID NO: 6 - DNA, 22 bp, Artificial Sequence
  Description of Artificial Sequence: Synthetic DNA
atcctcctcattcacccagatc

SEQ ID NO: 7 - DNA, 19 bp, Artificial Sequence
  Description of Artificial Sequence: Synthetic DNA
tggcacctcacctgcgaag

SEQ ID NO: 8 - DNA, 20 bp, Artificial Sequence
  Description of Artificial Sequence: Synthetic DNA
gcagaatggccactgctttg

SEQ ID NO: 9 - DNA, 19 bp, Artificial Sequence
  Description of Artificial Sequence: Synthetic DNA
tcgcacatgccgtgacttg

SEQ ID NO: 10 - DNA, 24 bp, Artificial Sequence
  Description of Artificial Sequence: Synthetic DNA
gatagcatccatagtgcatccttg

SEQ ID NO: 11 - DNA, 21 bp, Artificial Sequence
  Description of Artificial Sequence: Synthetic DNA
gccaggaatttgacgaagtca

SEQ ID NO: 12 - DNA, 22 bp, Artificial Sequence
  Description of Artificial Sequence: Synthetic DNA
cccatttctgcacatgtaccag

SEQ ID NO: 13 - DNA, 21 bp, Artificial Sequence
  Description of Artificial Sequence: Synthetic DNA
ctggtgagaagggtgagaaag

SEQ ID NO: 14 - DNA, 22 bp, Artificial Sequence
  Description of Artificial Sequence: Synthetic DNA
gtttcaccgatgtctcccttag